European Patent Specification EP 3 778 920 B1, published February 7, 2024. Title: Method of 3-dimensional nucleic acid imaging diagnosis of biological tissue using isothermal nucleic acid amplification. Applicant: BINAREE Inc. The sequence listing filed with the application follows.

SEQUENCE LISTING (16 sequences)

SEQ ID NO: 1 - DNA, 18 bp, Artificial Sequence
  Thy1-A F3 primer
gggagtccagaatccaag

SEQ ID NO: 2 - DNA, 16 bp, Artificial Sequence
  Thy1-B B3 primer
cgtgtgctcgggtatc

SEQ ID NO: 3 - DNA, 35 bp, Artificial Sequence
  Thy1-C FIP primer
tggtcaccttctgccctccttggcaccatgaaccc

SEQ ID NO: 4 - DNA, 34 bp, Artificial Sequence
  Thy1-D BIP primer
cttcgcctggactgcctgcttcctcttctctcgg

SEQ ID NO: 5 - DNA, 22 bp, Artificial Sequence
  Thy1-E LF primer
caagactgagagcaggagagcg

SEQ ID NO: 6 - DNA, 22 bp, Artificial Sequence
  Thy1-F LB primer
tccatccagcatgagttcagcc

SEQ ID NO: 7 - DNA, 42 bp, Artificial Sequence
  Thy1-HEX Fluorescent primer
caccaccctcccgtgggcggcaagactgagagcaggagagcg

SEQ ID NO: 8 - DNA, 20 bp, Artificial Sequence
  Thy-1-BHQ1 quencher primer
ccgcccacgggagggtggtg

SEQ ID NO: 9 - DNA, 20 bp, Artificial Sequence
  gad67-A F3 primer
gcaagacatttgatcgctcc

SEQ ID NO: 10 - DNA, 18 bp, Artificial Sequence
  gad67-B B3 primer
gagaacaaacacgggtgc

SEQ ID NO: 11 - DNA, 36 bp, Artificial Sequence
  gad67-C FIP primer
tgctccagagactcggggatttccaccacccacacc

SEQ ID NO: 12 - DNA, 36 bp, Artificial Sequence
  gad67-D BIP primer
cgcacaggtcaccctcgatgtcagccattcaccagc

SEQ ID NO: 13 - DNA, 18 bp, Artificial Sequence
  gad67-E LF primer
gccttccatgccttccag

SEQ ID NO: 14 - DNA, 21 bp, Artificial Sequence
  gad67-F LB primer
accagctctctactggtttgg

SEQ ID NO: 15 - DNA, 38 bp, Artificial Sequence
  gad67-Cy5 Fluorescent primer
gccacagccctctcccgccggccttccatgccttccag

SEQ ID NO: 16 - DNA, 20 bp, Artificial Sequence
  gad67-BHQ3 quencher primer
cggcgggagagggctgtggc